European Patent Application EP 4 696 712 A1, published February 18, 2026. Title: ANTI-DAT ANTIBODIES AND COMPOSITIONS THEREOF. Applicant: China Medical University. Application TW. The sequence listing filed with the application follows.

SEQUENCE LISTING (6 sequences)

SEQ ID NO: 1 - DNA, 798 bp, synthetic construct
  source 1..798: mol_type = other DNA
agcgctatggaccaagtgaagctggagcagagcggcgccgagctgatgaagcccggcgctagcgtgaagatcagctgcaaggccaccggctacaagttcagcagcaactggatcgagtgggtgaagcagagacccggccacggcctggagtggatcggcgagatcctgcccggaagcggtagcacgaattacaacgagaagttcaagggcaaggccaccttcaccgccgacacaagcagcaacaccgcctacatgcagctgagcagcctgacaagcgaggacagcgccgtgtactactgcgctagaagaagaacctactacggcaacttcttcgacagctggggccaaggcaccaccctgaccgtgagcagtgccaaaactacccctcctagtgtctatggtggagggggtagcggcggggggggctccgggggcggtggaagcgacatcgtgatgacacagagccccgctagcctgagcgtgagcgtgggcgagaccgtgaccatcacctgcagagctagcgagaacatctacagcaacctggcctggtatcagcagaagcaaggcaagagccctcagctgctggtgtacgccgccaccaacctggccgacggcgtgcctagcagattcagcggcagcggcagcgggacgcagtacagcctgaagatcaacagcctgcagagcgaggacttcggcagctactactgtcagcacttctggggcaccccctggaccttcggcggcggcaccaagctggagatcaagagagccgacgccgcccccaccgtgagcggatcc

SEQ ID NO: 2 - DNA, 360 bp, synthetic construct
  source 1..360: mol_type = other DNA
caggtgcagctgcaggagagcggcggcggcctggtgcaggccggcggcagcctgaggctgagctgcgccgccagcggcaggaccttcagcagctacgtgatgggctggttcaggcaggcccccggcaaggagagggagttcgtggccgccatcaacagcggcgacggcaggaccaactacgccgacagcgtgaagggcaggttcaccatcagcagggacaacgccaagaacaccgtgtacctgcagatgaacagcctgaagcccgaggacaccgccgtgtactactgcgccgccaggaggtaccccctgggcgacctgtacaactactggggccagggcacccaggtgaccgtgagcagc

SEQ ID NO: 3 - DNA, 732 bp, synthetic construct
  source 1..732: mol_type = other DNA
atggccgtggagggcggcatgaagtgcgtgaagttcctgctgtacgtgctgctgctggccttctgcgcctgtgccgtaggccttatcgccgttggcgtgggtgcgcagctggtcctttctcagaccataatccaaggagccacccccggcagcctgctgcccgtggtgatcatcgctgtgggggtcttcctgttcctggtggccttcgtgggctgctgcggcgcctgcaaggagaactactgcctgatgatcaccttcgccatcttcctgagcctgatcatgctggtggaggtggccgccgccatcgccggctacgtgttcagagacaaggtgatgagcgagttcaacaacaacttcagacagcagatggagaactaccccaagaacaaccacaccgccagcgctggatccagcatcctggacagaatgcaagccgacttcaagtgctgcggcgccgccaactacaccgactgggagaagatccctagcatgagcaagaacagagtgcccgacagctgctgcatcaacgtgaccgtgggctgcggcatcaacttcaacgagaaggccatccacaaggagggctgcgtggagaagatcggtggctggctgcgcaagaacgttctggtggtggccgccgccgccttaggcatcgccttcgtggaggtgctgggtatcgtgttcgcctgctgcctggtgaagagcatcagatcccaccaccaccaccaccactga

SEQ ID NO: 4 - DNA, 1092 bp, synthetic construct
  source 1..1092: mol_type = other DNA
atggccgtggagggcggcatgaagtgcgtgaagttcctgctgtacgtgctgctgctggccttctgcgcctgtgccgtaggccttatcgccgttggcgtgggtgcgcagctggtcctttctcagaccataatccaaggagccacccccggcagcctgctgcccgtggtgatcatcgctgtgggggtcttcctgttcctggtggccttcgtgggctgctgcggcgcctgcaaggagaactactgcctgatgatcaccttcgccatcttcctgagcctgatcatgctggtggaggtggccgccgccatcgccggctacgtgttcagagacaaggtgatgagcgagttcaacaacaacttcagacagcagatggagaactaccccaagaacaaccacaccgccagcgctcaggtgcagctgcaggagagcggcggcggcctggtgcaggccggcggcagcctgaggctgagctgcgccgccagcggcaggaccttcagcagctacgtgatgggctggttcaggcaggcccccggcaaggagagggagttcgtggccgccatcaacagcggcgacggcaggaccaactacgccgacagcgtgaagggcaggttcaccatcagcagggacaacgccaagaacaccgtgtacctgcagatgaacagcctgaagcccgaggacaccgccgtgtactactgcgccgccaggaggtaccccctgggcgacctgtacaactactggggccagggcacccaggtgaccgtgagcagcggatccagcatcctggacagaatgcaagccgacttcaagtgctgcggcgccgccaactacaccgactgggagaagatccctagcatgagcaagaacagagtgcccgacagctgctgcatcaacgtgaccgtgggctgcggcatcaacttcaacgagaaggccatccacaaggagggctgcgtggagaagatcggtggctggctgcgcaagaacgttctggtggtggccgccgccgccttaggcatcgccttcgtggaggtgctgggtatcgtgttcgcctgctgcctggtgaagagcatcagatcccaccaccaccaccaccactga

SEQ ID NO: 5 - DNA, 1002 bp, synthetic construct
  source 1..1002: mol_type = other DNA
atggccgtggagggcggcatgaagtgcgtgaagttcctgctgtacgtgctgctgctggccttctgcgcctgtgccgtaggccttatcgccgttggcgtgggtgcgcagctggtcctttctcagaccataatccaaggagccacccccggcagcctgctgcccgtggtgatcatcgctgtgggggtcttcctgttcctggtggccttcgtgggctgctgcggcgcctgcaaggagaactactgcctgatgatcaccttcgccatcttcctgagcctgatcatgctggtggaggtggccgccgccatcgccggctacgtgttcagagacaaggtgatgagcgagttcaacaacaacttcagacagcagatggagaactaccccaagaacaaccacaccgcctgcagagctagcgagaacatctacagcaacctggcctggtatcagcagaagcaaggcaagagccctcagctgctggtgtacgccgccaccaacctggccgacggcgtgcctagcagattcagcggcagcggcagcgggacgcagtacagcctgaagatcaacagcctgcagagcgaggacttcggcagctactactgtcagcacttctggggcaccccctggaccttcggcggcggcaccaagctggagatcaagagagccgacgccgcccccaccgtgagcggatccagcatcctggacagaatgcaagccgacttcaagtgctgcggcgccgccaactacaccgactgggagaagatccctagcatgagcaagaacagagtgcccgacagctgctgcatcaacgtgaccgtgggctgcggcatcaacttcaacgagaaggccatccacaaggagggctgcgtggagaagatcggtggctggctgcgcaagaacgttctggtggtggccgccgccgccttaggcatcgccttcgtggaggtgctgggtatcgtgttcgcctgctgcctggtgaagagcatcagatccggctatgaggtaatg

SEQ ID NO: 6 - DNA, 1512 bp, synthetic construct
  source 1..1512: mol_type = other DNA
atggccgtggagggcggcatgaagtgcgtgaagttcctgctgtacgtgctgctgctggccttctgcgcctgtgccgtaggccttatcgccgttggcgtgggtgcgcagctggtcctttctcagaccataatccaaggagccacccccggcagcctgctgcccgtggtgatcatcgctgtgggggtcttcctgttcctggtggccttcgtgggctgctgcggcgcctgcaaggagaactactgcctgatgatcaccttcgccatcttcctgagcctgatcatgctggtggaggtggccgccgccatcgccggctacgtgttcagagacaaggtgatgagcgagttcaacaacaacttcagacagcagatggagaactaccccaagaacaaccacaccgccagcgctatggaccaagtgaagctggagcagagcggcgccgagctgatgaagcccggcgctagcgtgaagatcagctgcaaggccaccggctacaagttcagcagcaactggatcgagtgggtgaagcagagacccggccacggcctggagtggatcggcgagatcctgcccggaagcggtagcacgaattacaacgagaagttcaagggcaaggccaccttcaccgccgacacaagcagcaacaccgcctacatgcagctgagcagcctgacaagcgaggacagcgccgtgtactactgcgctagaagaagaacctactacggcaacttcttcgacagctggggccaaggcaccaccctgaccgtgagcagtgccaaaactacccctcctagtgtctatggtggagggggtagcggcggggggggctccgggggcggtggaagcgacatcgtgatgacacagagccccgctagcctgagcgtgagcgtgggcgagaccgtgaccatcacctgcagagctagcgagaacatctacagcaacctggcctggtatcagcagaagcaaggcaagagccctcagctgctggtgtacgccgccaccaacctggccgacggcgtgcctagcagattcagcggcagcggcagcgggacgcagtacagcctgaagatcaacagcctgcagagcgaggacttcggcagctactactgtcagcacttctggggcaccccctggaccttcggcggcggcaccaagctggagatcaagagagccgacgccgcccccaccgtgagcggatccagcatcctggacagaatgcaagccgacttcaagtgctgcggcgccgccaactacaccgactgggagaagatccctagcatgagcaagaacagagtgcccgacagctgctgcatcaacgtgaccgtgggctgcggcatcaacttcaacgagaaggccatccacaaggagggctgcgtggagaagatcggtggctggctgcgcaagaacgttctggtggtggccgccgccgccttaggcatcgccttcgtggaggtgctgggtatcgtgttcgcctgctgcctggtgaagagcatcagatccggctatgaggtaatg